European Patent Specification EP 3 431 507 B1, published November 22, 2023. Title: NERVE GROWTH FACTOR FUSION PROTEIN, PREPARATION METHOD AND USE THEREOF. Applicant: STAIDSON(BEIJING) BIOPHARMACEUTICALS CO.,LTD. The sequence listing filed with the application follows.

SEQUENCE LISTING (45 sequences)

SEQ ID NO: 1 - protein, 241 aa, Homo sapiens, Human nerve growth factor
MTMLFYTLITAFLIGIQAEPHSESNVPAGHTIPQVHWTKLQHSLDTALRRARSAPAAAIAARVAGQTRNITVDPRLFKKRRLRSPRVLFSTQPPREAADTQDLDFEVGGAAPFNRTHRSKRSSSHPIFHRGEFSVCDSVSVWVGDKTTATDIKGKEVMVLGEVNINNSVFKQYFFETKCRDPNPVDSGCRGIDSKHWNSYCTTTHTFVKALTMDGKQAAWRFIRIDTACVCVLSRKAVRRA

SEQ ID NO: 2 - protein, 241 aa, Homo sapiens, NGF mutant F12E
MTMLFYTLITAFLIGIQAEPHSESNVPAGHTIPQVHWTKLQHSLDTALRRARSAPAAAIAARVAGQTRNITVDPRLFKKRRLRSPRVLFSTQPPREAADTQDLDFEVGGAAPFNRTHRSKRSSSHPIFHRGEESVCDSVSVWVGDKTTATDIKGKEVMVLGEVNINNSVFKQYFFETKCRDPNPVDSGCRGIDSKHWNSYCTTTHTFVKALTMDGKQAAWRFIRIDTACVCVLSRKAVRRA

SEQ ID NO: 3 - DNA, 723 bp, Homo sapiens, nucleotide sequence of β-NGF
atgaccatgttgttctacactctgatcacagcttttctgatcggcatacaggcggaaccacactcagagagcaatgtccctgcaggacacaccatcccccaagtccactggactaaacttcagcattcccttgacactgcccttcgcagagcccgcagcgccccggcagcggcgatagctgcacgcgtggcggggcagacccgcaacattactgtggaccccaggctgtttaaaaagcggcgactccgttcaccccgtgtgctgtttagcacccagcctccccgtgaagctgcagacactcaggatctggacttcgaggtcggtggtgctgcccccttcaacaggactcacaggagcaagcggtcatcatcccatcccatcttccacaggggcgaattctcggtgtgtgacagtgtcagcgtgtgggttggggataagaccaccgccacagacatcaagggcaaggaggtgatggtgttgggagaggtgaacattaacaacagtgtattcaaacagtacttttttgagaccaagtgccgggacccaaatcccgttgacagcgggtgccggggcattgactcaaagcactggaactcatattgtaccacgactcacacctttgtcaaggcgctgaccatggatggcaagcaggctgcctggcggtttatccggatagatacggcctgtgtgtgtgtgctcagcaggaaggctgtgagaagagcc

SEQ ID NO: 4 - DNA, 723 bp, Homo sapiens, nucleotide sequence of NGF mutant F12E
atgaccatgttgttctacactctgatcacagcttttctgatcggcatacaggcggaaccacactcagagagcaatgtccctgcaggacacaccatcccccaagtccactggactaaacttcagcattcccttgacactgcccttcgcagagcccgcagcgccccggcagcggcgatagctgcacgcgtggcggggcagacccgcaacattactgtggaccccaggctgtttaaaaagcggcgactccgttcaccccgtgtgctgtttagcacccagcctccccgtgaagctgcagacactcaggatctggacttcgaggtcggtggtgctgcccccttcaacaggactcacaggagcaagcggtcatcatcccatcccatcttccacaggggcgaagagtcggtgtgtgacagtgtcagcgtgtgggttggggataagaccaccgccacagacatcaagggcaaggaggtgatggtgttgggagaggtgaacattaacaacagtgtattcaaacagtacttttttgagaccaagtgccgggacccaaatcccgttgacagcgggtgccggggcattgactcaaagcactggaactcatattgtaccacgactcacacctttgtcaaggcgctgaccatggatggcaagcaggctgcctggcggtttatccggatagatacggcctgtgtgtgtgtgctcagcaggaaggctgtgagaagagcc

SEQ ID NO: 5 - protein, 232 aa, Homo sapiens, Fc moiety of IgG1
EPKSCDKTHTCPPCPAPELLGGPSVFLFPPKPKDTLMISRTPEVTCVVVDVSHEDPEVKFNWYVDGVEVHNAKTKPREEQYNSTYRVVSVLTVLHQDWLNGKEYKCKVSNKALPAPIEKTISKAKGQPREPQVYTLPPSREEMTKNQVSLTCLVKGFYPSDIAVEWESNGQPENNYKTTPPVLDSDGSFFLYSKLTVDKSRWQQGNVFSCSVMHEALHNHYTQKSLSLSPGK

SEQ ID NO: 6 - DNA, 699 bp, Homo sapiens, nucleotide sequence of Fc moiety of IgG1
gagcccaaatcttgtgacaaaactcacacatgcccaccgtgcccagcacctgaactcctggggggaccgtcagtcttcctcttccccccaaaacccaaggacaccctcatgatctcccggacccctgaggtcacatgcgtggtggtggacgtgagccacgaagaccctgaggtcaagttcaactggtacgtggacggcgtggaggtgcataatgccaagacaaagccgcgggaggagcagtacaacagcacgtaccgtgtggtcagcgtcctcaccgtcctgcaccaggactggctgaatggcaaggagtacaagtgcaaggtctccaacaaagccctcccagcccccatcgagaaaaccatctccaaagccaaagggcagccccgagaaccacaggtgtacaccctgcccccatcccgggaggagatgaccaagaaccaggtcagcctgacctgcctggtcaaaggcttctatcccagcgacatcgccgtggagtgggagagcaatgggcagccggagaacaactacaagaccacgcctcccgtgctggactccgacggctccttcttcctctatagcaagctcaccgtggacaagagcaggtggcagcaggggaacgtcttctcatgctccgtgatgcatgaggctctgcacaaccactacacgcagaagagcctctccctgtccccgggtaaatga

SEQ ID NO: 7 - protein, 231 aa, Homo sapiens, analog of Fc moiety of IgG1
EPKSCDKTHTCPPCPAPPVAGPSVFLFPPKPKDTLMISRTPEVTCVVVDVSHEDPEVKFNWYVDGVEVHNAKTKPREEQYNSTYRVVSVLTVLHQDWLNGKEYKCKVSNKGLPSSIEKTISKAKGQPREPQVYTLPPSREEMTKNQVSLTCLVKGFYPSDIAVEWESNGQPENNYKTTPPVLDSDGSFFLYSKLTVDKSRWQQGNVFSCSVMHEALHNHYTQKSLSLSPGK

SEQ ID NO: 8 - DNA, 696 bp, Homo sapiens, nucleotide sequence of human IgG1-Fc
gagcccaaatcttgtgacaaaactcacacatgcccaccgtgcccagcacctccagtcgcaggaccgtcagtcttcctcttccccccaaaacccaaggacaccctcatgatctcccggacccctgaggtcacatgcgtggtggtggacgtgagccacgaagaccctgaggtcaagttcaactggtacgtggacggcgtggaggtgcataatgccaagacaaagccgcgggaggagcagtacaacagcacgtaccgtgtggtcagcgtcctcaccgtcctgcaccaggactggctgaatggcaaggagtacaagtgcaaggtctccaacaaaggcctcccatcctccatcgagaaaaccatctccaaagccaaagggcagccccgagaaccacaggtgtacaccctgcccccatcccgggaggagatgaccaagaaccaggtcagcctgacctgcctggtcaaaggcttctatcccagcgacatcgccgtggagtgggagagcaatgggcagccggagaacaactacaagaccacgcctcccgtgctggactccgacggctccttcttcctctatagcaagctcaccgtggacaagagcaggtggcagcaggggaacgtcttctcatgctccgtgatgcatgaggctctgcacaaccactacacgcagaagagcctctccctgtccccgggtaaatga

SEQ ID NO: 9 - DNA, 681 bp, Homo sapiens, nucleotide sequence of human IgG1-Fc
gacaaaactcacacatgcccaccgtgcccagcacctccagtcgcaggaccgtcagtcttcctcttccccccaaaacccaaggacaccctcatgatctcccggacccctgaggtcacatgcgtggtggtggacgtgagccacgaagaccctgaggtcaagttcaactggtacgtggacggcgtggaggtgcataatgccaagacaaagccgcgggaggagcagtacaacagcacgtaccgtgtggtcagcgtcctcaccgtcctgcaccaggactggctgaatggcaaggagtacaagtgcaaggtctccaacaaaggcctcccatcctccatcgagaaaaccatctccaaagccaaagggcagccccgagaaccacaggtgtacaccctgcccccatcccgggaggagatgaccaagaaccaggtcagcctgacctgcctggtcaaaggcttctatcccagcgacatcgccgtggagtgggagagcaatgggcagccggagaacaactacaagaccacgcctcccgtgctggactccgacggctccttcttcctctatagcaagctcaccgtggacaagagcaggtggcagcaggggaacgtcttctcatgctccgtgatgcatgaggctctgcacaaccactacacgcagaagagcctctccctgtccccgggtaaatga

SEQ ID NO: 10 - protein, 482 aa, Homo sapiens, nerve growth factor fusion protein
MTMLFYTLITAFLIGIQAEPHSESNVPAGHTIPQVHWTKLQHSLDTALRRARSAPAAAIAARVAGQTRNITVDPRLFKKRRLRSPRVLFSTQPPREAADTQDLDFEVGGAAPFNRTHRSKRSSSHPIFHRGEESVCDSVSVWVGDKTTATDIKGKEVMVLGEVNINNSVFKQYFFETKCRDPNPVDSGCRGIDSKHWNSYCTTTHTFVKALTMDGKQAAWRFIRIDTACVCVLSRKAVRRAGGGGSGGGGSGGGGSDKTHTCPPCPAPPVAGPSVFLFPPKPKDTLMISRTPEVTCVVVDVSHEDPEVKFNWYVDGVEVHNAKTKPREEQYNSTYRVVSVLTVLHQDWLNGKEYKCKVSNKGLPSSIEKTISKAKGQPREPQVYTLPPSREEMTKNQVSLTCLVKGFYPSDIAVEWESNGQPENNYKTTPPVLDSDGSFFLYSKLTVDKSRWQQGNVFSCSVMHEALHNHYTQKSLSLSPGK

SEQ ID NO: 11 - DNA, 1449 bp, Homo sapiens, nucleotide sequence of nerve growth factor fusion protein
atgaccatgttgttctacactctgatcacagcttttctgatcggcatacaggcggaaccacactcagagagcaatgtccctgcaggacacaccatcccccaagtccactggactaaacttcagcattcccttgacactgcccttcgcagagcccgcagcgccccggcagcggcgatagctgcacgcgtggcggggcagacccgcaacattactgtggaccccaggctgtttaaaaagcggcgactccgttcaccccgtgtgctgtttagcacccagcctccccgtgaagctgcagacactcaggatctggacttcgaggtcggtggtgctgcccccttcaacaggactcacaggagcaagcggtcatcatcccatcccatcttccacaggggcgaagagtcggtgtgtgacagtgtcagcgtgtgggttggggataagaccaccgccacagacatcaagggcaaggaggtgatggtgttgggagaggtgaacattaacaacagtgtattcaaacagtacttttttgagaccaagtgccgggacccaaatcccgttgacagcgggtgccggggcattgactcaaagcactggaactcatattgtaccacgactcacacctttgtcaaggcgctgaccatggatggcaagcaggctgcctggcggtttatccggatagatacggcctgtgtgtgtgtgctcagcaggaaggctgtgagaagagccggcggtggcggctccggcggtggcggctccggcggtggcggctccgacaaaactcacacatgcccaccgtgcccagcacctccagtcgcaggaccgtcagtcttcctcttccccccaaaacccaaggacaccctcatgatctcccggacccctgaggtcacatgcgtggtggtggacgtgagccacgaagaccctgaggtcaagttcaactggtacgtggacggcgtggaggtgcataatgccaagacaaagccgcgggaggagcagtacaacagcacgtaccgtgtggtcagcgtcctcaccgtcctgcaccaggactggctgaatggcaaggagtacaagtgcaaggtctccaacaaaggcctcccatcctccatcgagaaaaccatctccaaagccaaagggcagccccgagaaccacaggtgtacaccctgcccccatcccgggaggagatgaccaagaaccaggtcagcctgacctgcctggtcaaaggcttctatcccagcgacatcgccgtggagtgggagagcaatgggcagccggagaacaactacaagaccacgcctcccgtgctggactccgacggctccttcttcctctatagcaagctcaccgtggacaagagcaggtggcagcaggggaacgtcttctcatgctccgtgatgcatgaggctctgcacaaccactacacgcagaagagcctctccctgtccccgggtaaatga

SEQ ID NO: 12 - DNA, 690 bp, Homo sapiens, nucleotide sequence of human IgG4-Fc
gagtccaaatatggtcccccatgcccaccctgcccagcacctgaggctgcggggggaccatcagtcttcctgttccccccaaaacccaaggacactctcatgatctcccggacccctgaggtcacgtgcgtggtggtggacgtgagccaggaagaccccgaggtccagttcaactggtacgtggatggcgtggaggtgcataatgccaagacaaagccgcgggaggagcagttcaacagcacgtaccgtgtggtcagcgtcctcaccgtcctgcaccaggactggctgaacggcaaggagtacaagtgcaaggtctccaacaaaggcctcccgtcctccatcgagaaaaccatctccaaagccaaagggcagccccgagagccacaggtgtacaccctgcccccatcccaggaggagatgaccaagaaccaggtcagcctgacctgcctggtcaaaggcttctaccccagcgacatcgccgtggagtgggaaagcaatgggcagccggagaacaactacaagaccacgcctcccgtgctggactccgacggctccttcttcctctacagcaggctaaccgtggacaagagcaggtggcaggaggggaatgtcttctcatgctccgtgatgcatgaggctctgcacaaccactacacacagaagagcctctccctgtctctgggtaaataa

SEQ ID NO: 13 - protein, 120 aa, Homo sapiens, NGF mutant K32G
SSSHPIFHRGEFSVCDSVSVWVGDKTTATDIGGKEVMVLGEVNINNSVFKQYFFETKCRDPNPVDSGCRGIDSKHWNSYCTTTHTFVKALTMDGKQAAWRFIRIDTACVCVLSRKAVRRA

SEQ ID NO: 14 - protein, 120 aa, Homo sapiens, NGF mutant K32L
SSSHPIFHRGEFSVCDSVSVWVGDKTTATDILGKEVMVLGEVNINNSVFKQYFFETKCRDPNPVDSGCRGIDSKHWNSYCTTTHTFVKALTMDGKQAAWRFIRIDTACVCVLSRKAVRRA

SEQ ID NO: 15 - protein, 120 aa, Homo sapiens: NGF mutant K32Y
SSSHPIFHRGEFSVCDSVSVWVGDKTTATDIYGKEVMVLGEVNINNSVFKQYFFETKCRDPNPVDSGCRGIDSKHWNSYCTTTHTFVKALTMDGKQAAWRFIRIDTACVCVLSRKAVRRA

SEQ ID NO: 16 - protein, 120 aa, Homo sapiens: NGF mutant R59L
SSSHPIFHRGEFSVCDSVSVWVGDKTTATDIKGKEVMVLGEVNINNSVFKQYFFETKCLDPNPVDSGCRGIDSKHWNSYCTTTHTFVKALTMDGKQAAWRFIRIDTACVCVLSRKAVRRA

SEQ ID NO: 17 - protein, 120 aa, Homo sapiens: NGF mutant R59A
SSSHPIFHRGEFSVCDSVSVWVGDKTTATDIKGKEVMVLGEVNINNSVFKQYFFETKCADPNPVDSGCRGIDSKHWNSYCTTTHTFVKALTMDGKQAAWRFIRIDTACVCVLSRKAVRRA

SEQ ID NO: 18 - protein, 120 aa, Homo sapiens: NGF mutant D65A
SSSHPIFHRGEFSVCDSVSVWVGDKTTATDIKGKEVMVLGEVNINNSVFKQYFFETKCRDPNPVASGCRGIDSKHWNSYCTTTHTFVKALTMDGKQAAWRFIRIDTACVCVLSRKAVRRA

SEQ ID NO: 19 - protein, 120 aa, Homo sapiens: NGF mutant D65G
SSSHPIFHRGEFSVCDSVSVWVGDKTTATDIKGKEVMVLGEVNINNSVFKQYFFETKCRDPNPVGSGCRGIDSKHWNSYCTTTHTFVKALTMDGKQAAWRFIRIDTACVCVLSRKAVRRA

SEQ ID NO: 20 - protein, 120 aa, Homo sapiens: NGF mutant K74L
SSSHPIFHRGEFSVCDSVSVWVGDKTTATDIKGKEVMVLGEVNINNSVFKQYFFETKCRDPNPVDSGCRGIDSLHWNSYCTTTHTFVKALTMDGKQAAWRFIRIDTACVCVLSRKAVRRA

SEQ ID NO: 21 - protein, 120 aa, Homo sapiens: NGF mutant K88F
SSSHPIFHRGEFSVCDSVSVWVGDKTTATDIKGKEVMVLGEVNINNSVFKQYFFETKCRDPNPVDSGCRGIDSKHWNSYCTTTHTFVFALTMDGKQAAWRFIRIDTACVCVLSRKAVRRA

SEQ ID NO: 22 - protein, 120 aa, Homo sapiens: NGF mutant K88L
SSSHPIFHRGEFSVCDSVSVWVGDKTTATDIKGKEVMVLGEVNINNSVFKQYFFETKCRDPNPVDSGCRGIDSKHWNSYCTTTHTFVLALTMDGKQAAWRFIRIDTACVCVLSRKAVRRA

SEQ ID NO: 23 - protein, 120 aa, Homo sapiens: NGF mutant K88E
SSSHPIFHRGEFSVCDSVSVWVGDKTTATDIKGKEVMVLGEVNINNSVFKQYFFETKCRDPNPVDSGCRGIDSKHWNSYCTTTHTFVEALTMDGKQAAWRFIRIDTACVCVLSRKAVRRA

SEQ ID NO: 24 - protein, 120 aa, Homo sapiens: NGF mutant K88G
SSSHPIFHRGEFSVCDSVSVWVGDKTTATDIKGKEVMVLGEVNINNSVFKQYFFETKCRDPNPVDSGCRGIDSKHWNSYCTTTHTFVGALTMDGKQAAWRFIRIDTACVCVLSRKAVRRA

SEQ ID NO: 25 - protein, 120 aa, Homo sapiens: NGF mutant Q96E
SSSHPIFHRGEFSVCDSVSVWVGDKTTATDIKGKEVMVLGEVNINNSVFKQYFFETKCRDPNPVDSGCRGIDSKHWNSYCTTTHTFVKALTMDGKEAAWRFIRIDTACVCVLSRKAVRRA

SEQ ID NO: 26 - protein, 120 aa, Homo sapiens: NGF mutant R114V
SSSHPIFHRGEFSVCDSVSVWVGDKTTATDIKGKEVMVLGEVNINNSVFKQYFFETKCRDPNPVDSGCRGIDSKHWNSYCTTTHTFVKALTMDGKQAAWRFIRIDTACVCVLSVKAVRRA

SEQ ID NO: 27 - protein, 120 aa, Homo sapiens: NGF mutant R114F
SSSHPIFHRGEFSVCDSVSVWVGDKTTATDIKGKEVMVLGEVNINNSVFKQYFFETKCRDPNPVDSGCRGIDSKHWNSYCTTTHTFVKALTMDGKQAAWRFIRIDTACVCVLSFKAVRRA

SEQ ID NO: 28 - protein, 120 aa, Homo sapiens: NGF mutant R114G
SSSHPIFHRGEFSVCDSVSVWVGDKTTATDIKGKEVMVLGEVNINNSVFKQYFFETKCRDPNPVDSGCRGIDSKHWNSYCTTTHTFVKALTMDGKQAAWRFIRIDTACVCVLSGKAVRRA

SEQ ID NO: 29 - protein, 120 aa, Homo sapiens: NGF mutant R114L
SSSHPIFHRGEFSVCDSVSVWVGDKTTATDIKGKEVMVLGEVNINNSVFKQYFFETKCRDPNPVDSGCRGIDSKHWNSYCTTTHTFVKALTMDGKQAAWRFIRIDTACVCVLSLKAVRRA

SEQ ID NO: 30 - protein, 120 aa, Homo sapiens: NGF mutant F101A
SSSHPIFHRGEFSVCDSVSVWVGDKTTATDIKGKEVMVLGEVNINNSVFKQYFFETKCRDPNPVDSGCRGIDSKHWNSYCTTTHTFVKALTMDGKQAAWRAIRIDTACVCVLSRKAVRRA

SEQ ID NO: 31 - DNA, 30 bp, Artificial sequence of primer F1
atttgcggccgcgccaccatgaccatgttg

SEQ ID NO: 32 - DNA, 50 bp, Artificial sequence of primer R2
gagttttgtcacaagatttgggctcggctcttctcacagccttcctgctg

SEQ ID NO: 33 - DNA, 50 bp, Artificial sequence of primer F2
cagcaggaaggctgtgagaagagccgagcccaaatcttgtgacaaaactc

SEQ ID NO: 34 - DNA, 43 bp, Artificial sequence of primer R2
gattgtcgatcattactaaccggttcatttacccggggacagg

SEQ ID NO: 35 - DNA, 45 bp, Artificial sequence
ggcggtggcggctccggcggtggcggctccggcggtggcggctcc

SEQ ID NO: 36 - DNA, 51 bp, Artificial sequence of primer F1-2
gccctctagactcgagcggccgcgccaccatgaccatgttgttctacactc

SEQ ID NO: 37 - DNA, 41 bp, Artificial sequence of primer R1-2
cgccggagccgccaccgccggctcttctcacagccttcctg

SEQ ID NO: 38 - DNA, 41 bp, Artificial sequence of primer F2-2
caggaaggctgtgagaagagccggcggtggcggctccggcg

SEQ ID NO: 39 - DNA, 50 bp, Artificial sequence of primer R2-2
gattgtcgatcattactaaccggttcatttacccggggacagggagaggc

SEQ ID NO: 40 - DNA, 33 bp, Artificial sequence of primer F12E-F
ttccacaggggcgaagagtcggtgtgtgacagt

SEQ ID NO: 41 - DNA, 33 bp, Artificial sequence of primer F12E-R
actgtcacacaccgactcttcgcccctgtggaa

SEQ ID NO: 42 - DNA, 33 bp, Artificial sequence of primer 1F
gtctctgggtaaataaaccggttagtaatgatc

SEQ ID NO: 43 - DNA, 31 bp, Artificial sequence of primer 1R
gaccatatttggactcggctcttctcacagc

SEQ ID NO: 44 - DNA, 40 bp, Artificial sequence of primer PAA-F
ctgcccagcacctgaggctgcggggggaccatcagtcttc

SEQ ID NO: 45 - DNA, 40 bp, Artificial sequence of primer PAA-R
gaagactgatggtccccccgcagcctcaggtgctgggcag